European Patent Specification EP 3 947 378 B1, published November 13, 2024. Title: NOVEL COMPOUNDS AND PHARMACEUTICAL COMPOSITIONS THEREOF FOR THE TREATMENT OF INFLAMMATORY DISORDERS. Applicant: Galapagos NV. The sequence listing filed with the application follows.

SEQUENCE LISTING (4 sequences)

SEQ ID NO: 1 - protein, 21 aa, Artificial Sequence
  RIP140 peptide
CYGVASSHLKTLLKKSKVKDQ

SEQ ID NO: 2 - protein, 21 aa, Artificial Sequence
  Histone H3 peptide
ARTKQTARKSTGGKAPRKQLC

SEQ ID NO: 3 - protein, 13 aa, Artificial Sequence
  Histone H1-derived peptide
GGGPATPKKAKKL

SEQ ID NO: 4 - protein, 39 aa, Artificial Sequence
  PDKtide
KTFCGTPEYLAPEVRREPRILSEEEQEMFRDFDYIADWC